European Patent Application EP 4 733 314 A1, published April 29, 2026. Title: Novel fusion protein and use thereof. Applicant: SL BIGEN, Inc. Application WO. The sequence listing filed with the application follows.

SEQUENCE LISTING (61 sequences)

SEQ ID NO: 1 - protein, 31 aa, synthetic construct
  REGION 1..31: note = human GLP-1
HGEGTFTSDVSSYLEGQAAKEFIAWLVKGRG

SEQ ID NO: 2 - protein, 31 aa, synthetic construct
  REGION 1..31: note = human GLP-1
HAEGTFTSDVSSYLEGQAAKEFIAWLVKGRG

SEQ ID NO: 3 - protein, 39 aa, synthetic construct
  REGION 1..39: note = Exendin 3
HSDGTFTSDLSKQMEEEAVRLFIEWLKNGGPSSGAPPPS

SEQ ID NO: 4 - protein, 39 aa, synthetic construct
  REGION 1..39: note = Exendin 4
HGEGTFTSDLSKQMEEEAVRLFIEWLKNGGPSSGAPPPS

SEQ ID NO: 5 - protein, 39 aa, synthetic construct
  REGION 1..39: note = GLP-1/Exendin 4 hybrid
HGEGTFTSDVSSYLEGQAAKEFIAWLVKGGPSSGAPPPS

SEQ ID NO: 6 - protein, 44 aa, synthetic construct
  REGION 1..44: note = Lixisenatide
HGEGTFTSDLSKQMEEEAVRLFIEWLKNGGPSSGAPPSKKKKKK

SEQ ID NO: 7 - protein, 905 aa, synthetic construct
  REGION 1..905: note = Exendin 4-XTEN
HGEGTFTSDLSKQMEEEAVRLFIEWLKNGGPSSGAPPPSGGSPAGSPTSTEEGTSESATPESGPGTSTEPSEGSAPGSPAGSPTSTEEGTSTEPSEGSAPGTSTEPSEGSAPGTSESATPESGPGSEPATSGSETPGSEPATSGSETPGSPAGSPTSTEEGTSESATPESGPGTSTEPSEGSAPGTSTEPSEGSAPGSPAGSPTSTEEGTSTEPSEGSAPGTSTEPSEGSAPGTSESATPESGPGTSTEPSEGSAPGTSESATPESGPGSEPATSGSETPGTSTEPSEGSAPGTSTEPSEGSAPGTSESATPESGPGTSESATPESGPGSPAGSPTSTEEGTSESATPESGPGSEPATSGSETPGTSESATPESGPGTSTEPSEGSAPGTSTEPSEGSAPGTSTEPSEGSAPGTSTEPSEGSAPGTSTEPSEGSAPGTSTEPSEGSAPGSPAGSPTSTEEGTSTEPSEGSAPGTSESATPESGPGSEPATSGSETPGTSESATPESGPGSEPATSGSETPGTSESATPESGPGTSTEPSEGSAPGTSESATPESGPGSPAGSPTSTEEGSPAGSPTSTEEGSPAGSPTSTEEGTSESATPESGPGTSTEPSEGSAPGTSESATPESGPGSEPATSGSETPGTSESATPESGPGSEPATSGSETPGTSESATPESGPGTSTEPSEGSAPGSPAGSPTSTEEGTSESATPESGPGSEPATSGSETPGTSESATPESGPGSPAGSPTSTEEGSPAGSPTSTEEGTSTEPSEGSAPGTSESATPESGPGTSESATPESGPGTSESATPESGPGSEPATSGSETPGSEPATSGSETPGSPAGSPTSTEEGTSTEPSEGSAPGTSTEPSEGSAPGSEPATSGSETPGTSESATPESGPGTSTEPSEGSAPG

SEQ ID NO: 8 - protein, 645 aa, synthetic construct
  REGION 1..645: note = Albiglutide
HGEGTFTSDVSSYLEGQAAKEFIAWLVKGRHGEGTFTSDVSSYLEGQAAKEFIAWLVKGRDAHKSEVAHRFKDLGEENFKALVLIAFAQYLQQCPFEDHVKLVNEVTEFAKTCVADESAENCDKSLHTLFGDKLCTVATLRETYGEMADCCAKQEPERNECFLQHKDDNPNLPRLVRPEVDVMCTAFHDNEETFLKKYLYEIARRHPYFYAPELLFFAKRYKAAFTECCQAADKAACLLPKLDELRDEGKASSAKQRLKCASLQKFGERAFKAWAVARLSQRFPKAEFAEVSKLVTDLTKVHTECCHGDLLECADDRADLAKYICENQDSISSKLKECCEKPLLEKSHCIAEVENDEMPADLPSLAADFVESKDVCKNYAEAKDVFLGMFLYEYARRHPDYSVVLLLRLAKTYETTLEKCCAAADPHECYAKVFDEFKPLVEEPQNLIKQNCELFEQLGEYKFQNALLVRYTKKVPQVSTPTLVEVSRNLGKVGSKCCKHPEAKRMPCAEDYLSVVLNQLCVLHEKTPVSDRVTKCCTESLVNRRPCFSALEVDETYVPKEFNAETFTFHADICTLSEKERQIKKQTALVELVKHKPKATKEQLKAVMDDFAAFVEKCCKADDKETCFAEEGKKLVAASQAALGL

SEQ ID NO: 9 - protein, 31 aa, synthetic construct
  REGION 1..31: note = Liraglutide
HAEGTFTSDVSSYLEGQAAKEFIAWLVRGRG

SEQ ID NO: 10 - protein, 30 aa, synthetic construct
  REGION 1..30: note = Taspoglutide
  MOD_RES 2: note = METHYLATION,
  MOD_RES 29: note = METHYLATION,
HXEGTFTSDVSSYLEGQAAKEFIAWLVKXR

SEQ ID NO: 11 - protein, 108 aa, synthetic construct
  REGION 1..108: note = GLP-1 tandem repeat
HGEGTFTSDVSSYLEGQAAKEFIAWLVKGGPSSGAPPPSGGGGSGGGGSGGGGSGGGGSGGGGSGGGGSHGEGTFTSDVSSYLEGQAAKEFIAWLVKGGPSSGAPPPS

SEQ ID NO: 12 - protein, 215 aa, synthetic construct
  REGION 1..215: note = hybrid Fc region
SHTQPLGVFLFPPKPKDTLMISRTPEVTCVVVDVSQEDPEVQFNWYVDGVEVHNAKTKPREEQFNSTYRVVSVLTVLHQDWLNGKEYKCKVSNKGLPSSIEKTISKAKGQPREPQVYTLPPSQEEMTKNQVSLTCLVKGFYPSDIAVEWESNGQPENNYKTTPPVLDSDGSFFLYSRLTVDKSRWQEGNVFSCSVMHEALHNHYTQKSLSLSLGK

SEQ ID NO: 13 - protein, 215 aa, synthetic construct
  REGION 1..215: note = hybrid Fc hole
SHTQPLGVFLFPPKPKDTLMISRTPEVTCVVVDVSQEDPEVQFNWYVDGVEVHNAKTKPREEQFNSTYRVVSVLTVLHQDWLNGKEYKCKVSNKGLPSSIEKTISKAKGQPREPQVCTLPPSQEEMTKNQVSLSCAVKGFYPSDIAVEWESNGQPENNYKTTPPVLDSDGSFFLVSRLTVDKSRWQEGNVFSCSVMHEALHNHYTQKSLSLSLGK

SEQ ID NO: 14 - protein, 215 aa, synthetic construct
  REGION 1..215: note = hybrid Fc knob
SHTQPLGVFLFPPKPKDTLMISRTPEVTCVVVDVSQEDPEVQFNWYVDGVEVHNAKTKPREEQFNSTYRVVSVLTVLHQDWLNGKEYKCKVSNKGLPSSIEKTISKAKGQPREPQVYTLPPCQEEMTKNQVSLWCLVKGFYPSDIAVEWESNGQPENNYKTTPPVLDSDGSFFLYSRLTVDKSRWQEGNVFSCSVMHEALHNHYTQKSLSLSLGK

SEQ ID NO: 15 - protein, 215 aa, synthetic construct
  REGION 1..215: note = hybrid Fc knob
SHTQPLGVFLFPPKPKDQLMISRTPEVTCVVVDVSQEDPEVQFNWYVDGVEVHNAKTKPREEQFNSTYRVVSVLTVLHQDWLNGKEYKCKVSNKGLPSSIEKTISKAKGQPREPQVYTLPPCQEEMTKNQVSLWCLVKGFYPSDIAVEWESNGQPENNYKTTPPVLDSDGSFFLYSRLTVDKSRWQEGNVFSCSVLHEALHNHYTQKSLSLSLGK

SEQ ID NO: 16 - protein, 215 aa, synthetic construct
  REGION 1..215: note = hybrid Fc hole
SHTQPLGVFLFPPKPKDQLMISRTPEVTCVVVDVSQEDPEVQFNWYVDGVEVHNAKTKPREEQFNSTYRVVSVLTVLHQDWLNGKEYKCKVSNKGLPSSIEKTISKAKGQPREPQVCTLPPSQEEMTKNQVSLSCAVKGFYPSDIAVEWESNGQPENNYKTTPPVLDSDGSFFLVSRLTVDKSRWQEGNVFSCSVLHEALHNHYTQKSLSLSLGK

SEQ ID NO: 17 - protein, 33 aa, synthetic construct
  REGION 1..33: note = human GLP-2 mutant (A2G)
HGDGSFSDEMNTILDNLAARDFINWLIQTKITD

SEQ ID NO: 18 - protein, 33 aa, synthetic construct
  REGION 1..33: note = human GLP-2 wild type
HADGSFSDEMNTILDNLAARDFINWLIQTKITD

SEQ ID NO: 19 - protein, 33 aa, synthetic construct
  REGION 1..33: note = human GLP-2 mutant (A2G, N16G, L17Q)
HGDGSFSDEMNTILDGQAARDFINWLIQTKITD

SEQ ID NO: 20 - protein, 33 aa, synthetic construct
  REGION 1..33: note = human GLP-2 mutant (A2G, L17Q)
HGDGSFSDEMNTILDNQAARDFINWLIQTKITD

SEQ ID NO: 21 - protein, 39 aa, synthetic construct
  REGION 1..39: note = Glepaglutide
HGEGTFSSELATILDALAARDFIAWLIATKITDKKKKKK

SEQ ID NO: 22 - protein, 42 aa, synthetic construct
  REGION 1..42: note = GLP-2 analogue 10
  MOD_RES 11: note = linked with a lipidated cross-linker via thiol groups of 11th and18th amino acids, cystein
  MOD_RES 18: note = linked with a lipidated cross-linker via thiol groups of 11th and18th amino acids, cystein
HGDGSFSDEMCTILDNLCARDFINWLIQTKITDPSSGAPPPS

SEQ ID NO: 23 - protein, 287 aa, synthetic construct
  REGION 1..287: note = first fusion protein of bispecific fusion protein containingGLP-1 analogue
HGEGTFTSDVSSYLEGQAAKEFIAWLVKGGPSSGAPPPSGGGGSGGGGSGGGGSEKEKEEQEERTHTCPPCPSHTQPLGVFLFPPKPKDQLMISRTPEVTCVVVDVSQEDPEVQFNWYVDGVEVHNAKTKPREEQFNSTYRVVSVLTVLHQDWLNGKEYKCKVSNKGLPSSIEKTISKAKGQPREPQVYTLPPCQEEMTKNQVSLWCLVKGFYPSDIAVEWESNGQPENNYKTTPPVLDSDGSFFLYSRLTVDKSRWQEGNVFSCSVLHEALHNHYTQKSLSLSLGK

SEQ ID NO: 24 - protein, 309 aa, synthetic construct
  REGION 1..309: note = first fusion protein of bispecific fusion protein containingGLP-1 analogue
HGEGTFTSDVSSYLEGQAAKEFIAWLVKGGPSSGAPPPSGGGGSGGGGSGGGGSAKNTTAPATTRNTTRGGEEKKKEKEKEEQEERTHTCPPCPSHTQPLGVFLFPPKPKDQLMISRTPEVTCVVVDVSQEDPEVQFNWYVDGVEVHNAKTKPREEQFNSTYRVVSVLTVLHQDWLNGKEYKCKVSNKGLPSSIEKTISKAKGQPREPQVYTLPPCQEEMTKNQVSLWCLVKGFYPSDIAVEWESNGQPENNYKTTPPVLDSDGSFFLYSRLTVDKSRWQEGNVFSCSVLHEALHNHYTQKSLSLSLGK

SEQ ID NO: 25 - protein, 353 aa, synthetic construct
  REGION 1..353: note = first fusion protein of bispecific fusion protein containingGLP-1 analogue
HGEGTFTSDVSSYLEGQAAKEFIAWLVKGGPSSGAPPPSGGGGSGGGGSGGGGSGGGGSGGGGSGGGGSHGEGTFTSDVSSYLEGQAAKEFIAWLVKGGPSSGAPPPSGGGGSGGGGSGGGGSEPKSSDKTHTCPPCPSHTQPLGVFLFPPKPKDQLMISRTPEVTCVVVDVSQEDPEVQFNWYVDGVEVHNAKTKPREEQFNSTYRVVSVLTVLHQDWLNGKEYKCKVSNKGLPSSIEKTISKAKGQPREPQVYTLPPCQEEMTKNQVSLWCLVKGFYPSDIAVEWESNGQPENNYKTTPPVLDSDGSFFLYSRLTVDKSRWQEGNVFSCSVLHEALHNHYTQKSLSLSLGK

SEQ ID NO: 26 - protein, 281 aa, synthetic construct
  REGION 1..281: note = second fusion protein of bispecific fusion protein containingGLP-2 analogue
HGDGSFSDEMNTILDNLAARDFINWLIQTKITDGGGGSGGGGSGGGGSEKEKEEQEERTHTCPPCPSHTQPLGVFLFPPKPKDQLMISRTPEVTCVVVDVSQEDPEVQFNWYVDGVEVHNAKTKPREEQFNSTYRVVSVLTVLHQDWLNGKEYKCKVSNKGLPSSIEKTISKAKGQPREPQVCTLPPSQEEMTKNQVSLSCAVKGFYPSDIAVEWESNGQPENNYKTTPPVLDSDGSFFLVSRLTVDKSRWQEGNVFSCSVLHEALHNHYTQKSLSLSLGK

SEQ ID NO: 27 - protein, 304 aa, synthetic construct
  REGION 1..304: note = second fusion protein of bispecific fusion protein containingGLP-2 analogue
HGDGSFSDEMNTILDNLAARDFINWLIQTKITDGGGGGSGGGGSGGGGSAKNTTAPATTRNTTRGGEEKKKEKEKEEQEERTHTCPPCPSHTQPLGVFLFPPKPKDQLMISRTPEVTCVVVDVSQEDPEVQFNWYVDGVEVHNAKTKPREEQFNSTYRVVSVLTVLHQDWLNGKEYKCKVSNKGLPSSIEKTISKAKGQPREPQVCTLPPSQEEMTKNQVSLSCAVKGFYPSDIAVEWESNGQPENNYKTTPPVLDSDGSFFLVSRLTVDKSRWQEGNVFSCSVLHEALHNHYTQKSLSLSLGK

SEQ ID NO: 28 - protein, 278 aa, synthetic construct
  REGION 1..278: note = second fusion protein of bispecific fusion protein containingGLP-2 analogue
HGDGSFSDEMNTILDGQAARDFINWLIQTKITDGGGGSGGGGSGGGGSEPKSSDKTHTCPPCPSHTQPLGVFLFPPKPKDQLMISRTPEVTCVVVDVSQEDPEVQFNWYVDGVEVHNAKTKPREEQFNSTYRVVSVLTVLHQDWLNGKEYKCKVSNKGLPSSIEKTISKAKGQPREPQVCTLPPSQEEMTKNQVSLSCAVKGFYPSDIAVEWESNGQPENNYKTTPPVLDSDGSFFLVSRLTVDKSRWQEGNVFSCSVLHEALHNHYTQKSLSLSLGK

SEQ ID NO: 29 - protein, 15 aa, synthetic construct
  REGION 1..15: note = linker peptide
EPKSSDKTHTCPPCP

SEQ ID NO: 30 - protein, 15 aa, synthetic construct
  REGION 1..15: note = linker peptide
EPKSCDKTHTCPPCP

SEQ ID NO: 31 - protein, 30 aa, synthetic construct
  REGION 1..30: note = linker peptide
GGGGSGGGGSGGGGSEPKSSDKTHTCPPCP

SEQ ID NO: 32 - protein, 30 aa, synthetic construct
  REGION 1..30: note = linker peptide
GGGGSGGGGSGGGGSEPKSCDKTHTCPPCP

SEQ ID NO: 33 - protein, 40 aa, synthetic construct
  REGION 1..40: note = linker peptide
AKATTAPATTRNTGRGGEEKKKEKEKEEQEERETKTPECP

SEQ ID NO: 34 - protein, 33 aa, synthetic construct
  REGION 1..33: note = linker peptide
GGGGSGGGGSGGGGSEKEKEEQEERTHTCPPCP

SEQ ID NO: 35 - protein, 55 aa, synthetic construct
  REGION 1..55: note = linker peptide
GGGGSGGGGSGGGGSAKNTTAPATTRNTTRGGEEKKKEKEKEEQEERTHTCPPCP

SEQ ID NO: 36 - protein, 20 aa, synthetic construct
  REGION 1..20: note = linker peptide
AAGSGGGGGSGGGGSGGGGS

SEQ ID NO: 37 - protein, 15 aa, synthetic construct
  REGION 1..15: note = linker peptide
GGGGSGGGGSGGGGS

SEQ ID NO: 38 - protein, 5 aa, synthetic construct
  REGION 1..5: note = linker peptide
GGSGG

SEQ ID NO: 39 - protein, 9 aa, synthetic construct
  REGION 1..9: note = linker peptide
GGSGGSGGS

SEQ ID NO: 40 - protein, 6 aa, synthetic construct
  REGION 1..6: note = linker peptide
GGGSGG

SEQ ID NO: 41 - protein, 5 aa, synthetic construct
  REGION 1..5: note = linker peptide unit sequence
GGGGS

SEQ ID NO: 42 - protein, 6 aa, synthetic construct
  REGION 1..6: note = linker peptide unit sequence
GSSGGS

SEQ ID NO: 43 - protein, 18 aa, synthetic construct
  REGION 1..18: note = linker peptide
KESGSVSSEQLAQFRSLD

SEQ ID NO: 44 - protein, 14 aa, synthetic construct
  REGION 1..14: note = linker peptide
EGKSSGSGSESKST

SEQ ID NO: 45 - protein, 12 aa, synthetic construct
  REGION 1..12: note = linker peptide
GSAGSAAGSGEF

SEQ ID NO: 46 - protein, 5 aa, synthetic construct
  REGION 1..5: note = linker peptide unit sequence
EAAAK

SEQ ID NO: 47 - protein, 12 aa, synthetic construct
  REGION 1..12: note = linker peptide
CRRRRRREAEAC

SEQ ID NO: 48 - protein, 46 aa, synthetic construct
  REGION 1..46: note = linker peptide
AEAAAKEAAAKEAAAKEAAAKALEAEAAAKEAAAKEAAAKEAAAKA

SEQ ID NO: 49 - protein, 8 aa, synthetic construct
  REGION 1..8: note = linker peptide
GGGGGGGG

SEQ ID NO: 50 - protein, 6 aa, synthetic construct
  REGION 1..6: note = linker peptide
GGGGGG

SEQ ID NO: 51 - protein, 13 aa, synthetic construct
  REGION 1..13: note = linker peptide
AEAAAKEAAAAKA

SEQ ID NO: 52 - protein, 5 aa, synthetic construct
  REGION 1..5: note = linker peptide
PAPAP

SEQ ID NO: 53 - protein, 17 aa, synthetic construct
  REGION 1..17: note = linker peptide
VSQTSKLTRAETVFPDV

SEQ ID NO: 54 - protein, 6 aa, synthetic construct
  REGION 1..6: note = linker peptide
PLGLWA

SEQ ID NO: 55 - protein, 10 aa, synthetic construct
  REGION 1..10: note = linker peptide
TRHRQPRGWE

SEQ ID NO: 56 - protein, 10 aa, synthetic construct
  REGION 1..10: note = linker peptide
AGNRVRRSVG

SEQ ID NO: 57 - protein, 8 aa, synthetic construct
  REGION 1..8: note = linker peptide
RRRRRRRR

SEQ ID NO: 58 - protein, 4 aa, synthetic construct
  REGION 1..4: note = linker peptide
GFLG

SEQ ID NO: 59 - protein, 31 aa, synthetic construct
  REGION 1..31: note = linker peptide
GSSGGSGSSGGSGGGDEADGSRGSQKAGVDE

SEQ ID NO: 60 - protein, 15 aa, synthetic construct
  REGION 1..15: note = linker peptide
GSTSGSGKPGSGEGS

SEQ ID NO: 61 - protein, 103 aa, synthetic construct
  REGION 1..103: note = IgG1 CH3 domain
EPQVYTLPPSRDELTKNQVSLTCLVKGFYPSDIAVEWESNGQPENNYKTTPPVLDSDGSFFLYSKLTVDKSRWQQGNVFSCSVMHEALHNHYTQKSLSLSPGK